European Patent Application EP 4 736 894 A1, published May 6, 2026. Title: Antimicrobial peptide-functionalized crosslinkable copolymer, crosslinked copolymer and hydrogel with antibacterial activity. Applicant: Universität Siegen, Körperschaft des öffentlichen Rechts. The sequence listing filed with the application follows.

SEQUENCE LISTING (30 sequences)

SEQ ID NO: 1 - protein, 24 aa, synthetic construct
  REGION 1..24: note = Synthetic antimicrobial peptide
LKRVWKRVFKLLKRYWRQLKKPVR

SEQ ID NO: 2 - protein, 24 aa, synthetic construct
  REGION 1..24: note = Synthetic antimicrobial peptide
LKRLYKRLAKLIKRLYRYLKKPVR

SEQ ID NO: 3 - protein, 24 aa, synthetic construct
  REGION 1..24: note = Synthetic antimicrobial peptide
LKRVWKAVFKLLKRYWRQLKKPVR

SEQ ID NO: 4 - protein, 24 aa, synthetic construct
  REGION 1..24: note = Synthetic antimicrobial peptide
IGKEFKRIVERIKRFLRELVRPLR

SEQ ID NO: 5 - protein, 15 aa, synthetic construct
  REGION 1..15: note = Synthetic antimicrobial peptide
LRCMCIKWWSGKHPK

SEQ ID NO: 6 - protein, 15 aa, synthetic construct
  REGION 1..15: note = Synthetic antimicrobial peptide
LRAMCIKWWSGKHPK

SEQ ID NO: 7 - protein, 19 aa, synthetic construct
  REGION 1..19: note = Synthetic antimicrobial peptide
GKWKLFKKAFKKFLKILAC

SEQ ID NO: 8 - protein, 24 aa, synthetic construct
  REGION 1..24: note = Synthetic antimicrobial peptide
LKKLWKRVFRIWKRIFRYLKRPVR

SEQ ID NO: 9 - protein, 24 aa, synthetic construct
  REGION 1..24: note = Synthetic antimicrobial peptide
LRRLWKRLVRIIKRIYRQLKRPVR

SEQ ID NO: 10 - protein, 24 aa, synthetic construct
  REGION 1..24: note = Synthetic antimicrobial peptide
LRRLYKRVFRLLKRWWRYLKRPVR

SEQ ID NO: 11 - protein, 24 aa, synthetic construct
  REGION 1..24: note = Synthetic antimicrobial peptide
LRRLWKRLVKILKRWFRYLRRPVR

SEQ ID NO: 12 - protein, 24 aa, synthetic construct
  REGION 1..24: note = Synthetic antimicrobial peptide
LRRLYKRVVKLWKRLFRQLRRPVR

SEQ ID NO: 13 - protein, 24 aa, synthetic construct
  REGION 1..24: note = Synthetic antimicrobial peptide
LKKLYKRVAKIWKRWIRYLKKPVR

SEQ ID NO: 14 - protein, 24 aa, synthetic construct
  REGION 1..24: note = Synthetic antimicrobial peptide
LKKLYKRLFKILKRILRYLRKPVR

SEQ ID NO: 15 - protein, 24 aa, synthetic construct
  REGION 1..24: note = Synthetic antimicrobial peptide
LKKLWKRLARLLKRFIRQLRRPVR

SEQ ID NO: 16 - protein, 24 aa, synthetic construct
  REGION 1..24: note = Synthetic antimicrobial peptide
LKKVYKRLARLLKRYIRYLRRPVR

SEQ ID NO: 17 - protein, 24 aa, synthetic construct
  REGION 1..24: note = Synthetic antimicrobial peptide
LKKVWKRVARLIKRWFRYLRRPVR

SEQ ID NO: 18 - protein, 24 aa, synthetic construct
  REGION 1..24: note = Synthetic antimicrobial peptide
LKKLYKRLFKLWKRLYRYLKKPVR

SEQ ID NO: 19 - protein, 24 aa, synthetic construct
  REGION 1..24: note = Synthetic antimicrobial peptide
LRRVYKRLARLIKRYLRQLKKPVR

SEQ ID NO: 20 - protein, 24 aa, synthetic construct
  REGION 1..24: note = Synthetic antimicrobial peptide
LRKLWKRVVKIWKRYLRQLRRPVR

SEQ ID NO: 21 - protein, 24 aa, synthetic construct
  REGION 1..24: note = Synthetic antimicrobial peptide
LRKLWKRLAKIIKRLYRYLRRPVR

SEQ ID NO: 22 - protein, 24 aa, synthetic construct
  REGION 1..24: note = Synthetic antimicrobial peptide
LKKVYKRVARLIKRLFRYLKRPVR

SEQ ID NO: 23 - protein, 24 aa, synthetic construct
  REGION 1..24: note = Synthetic antimicrobial peptide
LRRLWKRLVKLWKRFFRYLKKPVR

SEQ ID NO: 24 - protein, 24 aa, synthetic construct
  REGION 1..24: note = Synthetic antimicrobial peptide
LKKVWKRVFRILKRFLRYLKRPVR

SEQ ID NO: 25 - protein, 24 aa, synthetic construct
  REGION 1..24: note = Synthetic antimicrobial peptide
LRRVYKRLFRLWKRIIRQLRRPVR

SEQ ID NO: 26 - protein, 24 aa, synthetic construct
  REGION 1..24: note = Synthetic antimicrobial peptide
LKRLYKRVFRLLKRYYRQLRRPVR

SEQ ID NO: 27 - protein, 24 aa, synthetic construct
  REGION 1..24: note = Synthetic antimicrobial peptide
LKKLWKRLARLWKRIIRQLKKPVR

SEQ ID NO: 28 - protein, 24 aa, synthetic construct
  REGION 1..24: note = Synthetic antimicrobial peptide
LRRVWKRVARIIKRLYRYLKRPVR

SEQ ID NO: 29 - protein, 24 aa, synthetic construct
  REGION 1..24: note = Synthetic antimicrobial peptide
LKRLWKRLFKILKRYYRYLRRPVR

SEQ ID NO: 30 - protein, 24 aa, synthetic construct
  REGION 1..24: note = Synthetic antimicrobial peptide
LRRLWKRVFKIIKRLFRQLKKPVR